European Patent Application EP 4 737 568 A1, published May 6, 2026. Title: Novel CRISPR/Cas13 system and use thereof. Applicant: NSAGE INC. The sequence listing filed with the application follows.

SEQUENCE LISTING (87 sequences)

SEQ ID NO: 1 - protein, 921 aa, synthetic construct
  source 1..921: note = New Cas13 protein
VSKNDNIKSKAKALGLKSTFQVGDEVVMTSFGKGNKAIVEKIVRGTDVQSVPTEPNFSAEIEGKKFDLVGRAHIQTKSDNPQYSKKRTGDDMIGAKAALEKRFFGGTFDDNIHIQLAYNVLDIEKILSVHINNIVYTLNNIRRKDNAEDDDFIGYMSTRNDYDTFIEPRKHNISEDAAKSIDKSRASFEEYLQPPVKDCLHYFGNTFFAPREIEKTYTDNRGFERKKKVTVNSLIDEKEIYYIFALLGGLRQFCTHDNKSGRNWLYSLEENGINSDAKAVLDKYYNSAVARIDESFVDNASKTNFKLIFNAMDVSDEALQDNIAKAFYKFTVCKSFKNMGFSIKKLREQLLELPEYEGLKDKHYDSVRSKLYQIMDFVIYLSFKDEKFKKDNEEKINNIVNELRATLNEEDKGRVYASYAERMKSELKPAIARLKSDIDKIKDSRVKEFELDASVKYRLSKVVESVRLKDRATYFTKLIYLTTLFLDGKEINDLLTTLIHQFENIASFIDVMNDRGIDCRFSDGYKLFESSKQIAFELRNVNSFARMTRTSKDDENATHMMYIDAAEILGTDYTEEQIEEHLNLEKKRMIPGTKKADMNFRNFIINNVIKSSRFNYLVRYSNPKKIRALADNEGVIRFVLGELPDAQIDRYTLLCGFNPDADRQEKTDKLAKAITGLRFNDFENVKQGANTEGESQESIDKAQKQGLISLYLTVLYLLTKNLVYVNSRYFLAFHCLERDAQLLGSGAGHHEPYVALTQRFINEDKLNEHACEYLKTNIANSDEYTIRIFRNNAAHLSAVRNANLYIDKLKEFKSYYEIYHFLSQENIYGKYCVDKKYVTADENGSKTISVKISKDYCPQVYIDKSLEYFDKLNKYGTYCKDFTKALNSPFGYNLARYKNLSIEGLFDRNRPGDKGENTFED

SEQ ID NO: 2 - RNA, 37 nt, synthetic construct
  source 1..37: mol_type = other RNA; note = Direct Repeat of New Cas13 guide RNA
gaaacgtactacaccctttttgtaagggtctgaaacc

SEQ ID NO: 3 - RNA, 37 nt, synthetic construct
  source 1..37: mol_type = other RNA; note = Candidate sequence of Direct Repeat of new Cas13 guide RNA
ggtttcagacccttacaaaaagggtgtagtacgtttc

SEQ ID NO: 4 - DNA, 2766 bp, synthetic construct
  source 1..2766: mol_type = other DNA; note = DNA encoding Direct Repeat of new Cas13 protein
gtgagcaagaatgataacatcaaatccaaagcaaaagcacttggcttgaagtcaacgtttcaggttggcgacgaggtcgttatgacttctttcggtaaaggtaataaagccatcgttgaaaagattgtacgtggaaccgacgtgcagtctgttccgactgagccgaacttcagcgctgaaatcgaaggtaaaaaatttgaccttgtcggcagagctcatattcagacaaagtcggacaatcctcagtattcaaagaaaagaaccggcgacgatatgataggcgcaaaggcggcacttgaaaagagattcttcggcggtacgtttgacgacaatatacatattcagctcgcttacaatgttcttgatattgaaaagattctttctgtccatatcaacaatattgtttacacgcttaataacatacgaagaaaagacaacgctgaagatgacgattttatcggctatatgagtaccagaaacgactacgacacctttattgaaccgagaaagcacaacattagcgaagacgctgctaaaagcattgacaaatcaagagcctcgtttgaagagtatcttcagccgccggtaaaggattgtctgcattatttcggaaacaccttttttgctccccgtgagattgaaaagacatacacggataatcgcggctttgaaaggaagaaaaaagttaccgtaaactcgcttatagacgagaaggaaatatactatatttttgccctcctcggcggacttcgtcaattctgtacccatgacaacaaaagcggcagaaactggctttattctctcgaggaaaacggaataaactctgatgcaaaggcggtacttgacaagtactataattctgcagttgcaaggattgacgaaagctttgttgacaacgcatctaaaactaatttcaagctgatttttaatgcaatggatgtcagcgacgaagcgcttcaggacaatatagcaaaggcgttttacaagtttacggtttgtaagagctttaaaaacatgggcttttcaattaaaaagctccgtgaacagctgctcgaacttcctgaatatgaagggcttaaagataagcattacgattccgtgcgctcaaagctttatcagattatggacttcgttatttatctgagtttcaaagatgaaaagtttaagaaggataatgaagaaaagattaataatatcgttaacgaactccgtgcgaccttgaacgaagaggataaaggcagagtatatgcctcttatgccgaaaggatgaaatctgagcttaaaccggcaattgcacgccttaagtctgatattgacaaaattaaggacagcagggtgaaagagtttgaacttgatgcgtccgtaaaatatagactctcaaaggtcgtagaaagtgtgcgccttaaggatagggcaacatattttacaaagctcatatatctgactactctgttccttgacggcaaggagattaacgacctcctgactactcttattcatcagtttgagaatatcgcaagttttattgatgttatgaacgacagaggtattgattgccgtttttcggatggatataagctttttgaatcctcaaagcaaattgcgtttgagcttcgcaatgtcaatagctttgctcgtatgacaaggacctcaaaggatgacgaaaacgcaacgcatatgatgtatatagatgctgcagagattctcggcaccgattataccgaagagcagattgaggagcatcttaacctggaaaagaaaagaatgataccaggcacgaaaaaagcggatatgaacttccgtaactttataatcaataacgttataaagtcatcacgcttcaattatcttgtcagatattccaatcctaaaaaaatcagagcgctcgccgataacgagggtgtaatccgttttgtcctgggcgagttgccggatgcgcagattgaccgttatactttactttgcggcttcaatcccgatgccgaccggcaggaaaaaacggacaaacttgcaaaggcaattactggtttgaggtttaacgattttgaaaatgttaaacagggcgcaaatactgagggcgaatctcaggagtcaattgacaaggcacagaagcagggactgatttctttgtacttaaccgttctatatcttttgacaaagaatcttgtttatgtaaactcacgctattttcttgcattccattgtcttgagcgtgatgcgcagctgcttggaagcggtgctgggcatcatgagccttatgttgctcttactcagcgctttattaatgaagataagctcaatgagcatgcctgcgaatatcttaagaccaatattgcaaattcggatgaatatacaattagaatattccgcaataatgctgctcacttgagtgctgttagaaatgcaaatctgtatattgacaagttgaaggaatttaaatcgtactatgagatttatcatttcctttctcaagagaatatttacggtaaatattgcgttgataagaaatatgttacagccgatgaaaatggaagtaaaacaataagtgttaaaattagcaaggattattgtcctcaggtatatatcgacaagtcgcttgaatactttgacaagctcaataaatatggtacgtattgcaaggacttcacgaaggcactcaattcgccattcggctacaacctcgcaagatataagaatctgtctatcgagggcttgtttgaccgaaaccgtcccggagacaaaggtgagaacacgtttgaggactaa

SEQ ID NO: 5 - RNA, 969 nt, synthetic construct
  source 1..969: mol_type = other RNA; note = COVID-19, N-gene
tctgataatggaccccaaaatcagcgaaatgcaccccgcattacgtttggtggaccctcagattcaactggcagtaaccagaatggagaacgcagtggggcgcgatcaaaacaacgtcggccccaaggtttacccaataatactgcgtcttggttcaccgctctcactcaacatggcaaggaagaccttaaattccctcgaggacaaggcgttccaattaacaccaatagcagtccagatgaccaaattggctactaccgaagagctaccagacgaattcgtggtggtgacggtaaaatgaaagatctcagtccaagatggtatttctactacctaggaactgggccagaagctggactccctatggtgctaacaaagacggcatcatagggttgcaactgagggagccttgaatacaccaaaagatcacattggcacccgcaatcctgctaacaatgctgcaatcgtgctacaacttcctcaaggaacaacattgccaaaaggcttctacgcagaagggagcagaggcggcagtcaagcctcttctcgttcctcatcacgtagtcgcaacagttcaagaaattcaactccaggcagcagtaggggaacctcctgctagaatggctggcaatggcggtgatgctgctcttgctttgctgctgcttgacagattgaaccagcttgagagcaaaatgtctggtaaaggccaacaacaacaaggccaaactgtcactaagaaatctgctgctgaggcttctaagaagcctcggcaaaaacgtactgccactaaagcatacaatgtaacacaagctttcggcagacgtggtccagaacaaacccaaggaaattttggggaccaggaactaatcagacaaggaactgattacaaacattggccgcaaattgcacaatttgcccccagcgcttcagcgttcttcggaatgtcgcgcattggcatggaagaaaaaa

SEQ ID NO: 6 - RNA, 229 nt, synthetic construct
  source 1..229: mol_type = other RNA; note = COVID-19,E-gene
tactcattcgtttcggaagagacaggtacgttaatagttaatagcgtacttctttttcttgctttcgtggtattcttgctagttacactagccatccttactgcgcttcgattgtgtgcgtactgctgcaatattgttaacgtgagtcttgtaaaaccttctttttacgtttactctcgtgttaaaaatctgaattcttctagagttcctgatcttctggtctaaaaaa

SEQ ID NO: 7 - RNA, 57 nt, synthetic construct
  source 1..57: mol_type = other RNA; note = Guide RNA targeting N-gene, DR dir, PFS = C
ggtttcagacccttacaaaaagggtgtagtacgtttcggtccaccaaacgtaatgcg

SEQ ID NO: 8 - RNA, 57 nt, synthetic construct
  source 1..57: mol_type = other RNA; note = Guide RNA targeting N-gene, DR dir, PFS = A
ggtttcagacccttacaaaaagggtgtagtacgtttctctggttactgccagttgaa

SEQ ID NO: 9 - RNA, 57 nt, synthetic construct
  source 1..57: mol_type = other RNA; note = Guide RNA targeting N-gene, DR dir, PFS = T
ggtttcagacccttacaaaaagggtgtagtacgtttctttgcggccaatgtttgtaa

SEQ ID NO: 10 - RNA, 57 nt, synthetic construct
  source 1..57: mol_type = other RNA; note = Guide RNA targeting N-gene, DR dir, PFS = A
ggtttcagacccttacaaaaagggtgtagtacgtttcttggtgtattcaaggctccc

SEQ ID NO: 11 - RNA, 57 nt, synthetic construct
  source 1..57: mol_type = other RNA; note = Guide RNA targeting N-gene, DR dir, PFS = T
ggtttcagacccttacaaaaagggtgtagtacgtttcggattgcgggtgccaatgtg

SEQ ID NO: 12 - RNA, 57 nt, synthetic construct
  source 1..57: mol_type = other RNA; note = Guide RNA targeting N-gene, DR dir, PFS = A
ggtttcagacccttacaaaaagggtgtagtacgtttctgtagcacgattgcagcatt

SEQ ID NO: 13 - RNA, 57 nt, synthetic construct
  source 1..57: mol_type = other RNA; note = Guide RNA targeting N-gene, DR dir, PFS = A
ggtttcagacccttacaaaaagggtgtagtacgtttctctagcaggagaagttcccc

SEQ ID NO: 14 - RNA, 57 nt, synthetic construct
  source 1..57: mol_type = other RNA; note = Guide RNA targeting N-gene, DR dir, PFS = T
ggtttcagacccttacaaaaagggtgtagtacgtttctctgtcaagcagcagcaaag

SEQ ID NO: 15 - RNA, 57 nt, synthetic construct
  source 1..57: mol_type = other RNA; note = Guide RNA targeting N-gene, DR dir, PFS = T
ggtttcagacccttacaaaaagggtgtagtacgtttcgacattttgctctcaagctg

SEQ ID NO: 16 - RNA, 57 nt, synthetic construct
  source 1..57: mol_type = other RNA; note = Guide RNA targeting N-gene, DR rev, PFS = G
gaaacgtactacaccctttttgtaagggtctgaaacctggttactgccagttgaatc

SEQ ID NO: 17 - RNA, 58 nt, synthetic construct
  source 1..58: mol_type = other RNA; note = Guide RNA targeting N-gene, DR rev, PFS = G
gaaacgtactacaccctttttgtaagggtctgaaaccaggattgcgggtgccaatgtg

SEQ ID NO: 18 - RNA, 58 nt, synthetic construct
  source 1..58: mol_type = other RNA; note = Guide RNA targeting N-gene, DR rev, PFS = C
gaaacgtactacaccctttttgtaagggtctgaaaccttgtagcacgattgcagcatt

SEQ ID NO: 19 - RNA, 60 nt, synthetic construct
  source 1..60: mol_type = other RNA; note = Guide RNA targeting N-gene, DR rev, PFS = C
gaaacgtactacaccctttttgtaagggtctgaaacccaaattgtgcaatttgcggccaa

SEQ ID NO: 20 - RNA, 60 nt, synthetic construct
  source 1..60: mol_type = other RNA; note = Guide RNA targeting N-gene, DR rev, PFS = C
gaaacgtactacaccctttttgtaagggtctgaaaccgccaatgtttgtaatcagttcct

SEQ ID NO: 21 - RNA, 60 nt, synthetic construct
  source 1..60: mol_type = other RNA; note = Guide RNA targeting N-gene, DR rev, PFS = G
gaaacgtactacaccctttttgtaagggtctgaaaccttgtctgattagttcctggtccc

SEQ ID NO: 22 - RNA, 57 nt, synthetic construct
  source 1..57: mol_type = other RNA; note = Guide RNA targeting N-gene, DR rev, PFS = C
gaaacgtactacaccctttttgtaagggtctgaaaccggtccaccaaacgtaatgcg

SEQ ID NO: 23 - RNA, 57 nt, synthetic construct
  source 1..57: mol_type = other RNA; note = Guide RNA targeting N-gene, DR rev, PFS = A
gaaacgtactacaccctttttgtaagggtctgaaacctctggttactgccagttgaa

SEQ ID NO: 24 - RNA, 57 nt, synthetic construct
  source 1..57: mol_type = other RNA; note = Guide RNA targeting N-gene, DR rev, PFS = T
gaaacgtactacaccctttttgtaagggtctgaaacctttgcggccaatgtttgtaa

SEQ ID NO: 25 - RNA, 57 nt, synthetic construct
  source 1..57: mol_type = other RNA; note = Guide RNA targeting N-gene, DR rev, PFS = A
gaaacgtactacaccctttttgtaagggtctgaaaccttggtgtattcaaggctccc

SEQ ID NO: 26 - RNA, 57 nt, synthetic construct
  source 1..57: mol_type = other RNA; note = Guide RNA targeting N-gene, DR rev, PFS = T
gaaacgtactacaccctttttgtaagggtctgaaaccggattgcgggtgccaatgtg

SEQ ID NO: 27 - RNA, 57 nt, synthetic construct
  source 1..57: mol_type = other RNA; note = Guide RNA targeting N-gene, DR rev, PFS = A
gaaacgtactacaccctttttgtaagggtctgaaacctgtagcacgattgcagcatt

SEQ ID NO: 28 - RNA, 57 nt, synthetic construct
  source 1..57: mol_type = other RNA; note = Guide RNA targeting N-gene, DR rev, PFS = A
gaaacgtactacaccctttttgtaagggtctgaaacctctagcaggagaagttcccc

SEQ ID NO: 29 - RNA, 57 nt, synthetic construct
  source 1..57: mol_type = other RNA; note = Guide RNA targeting N-gene, DR rev, PFS = T
gaaacgtactacaccctttttgtaagggtctgaaacctctgtcaagcagcagcaaag

SEQ ID NO: 30 - RNA, 57 nt, synthetic construct
  source 1..57: mol_type = other RNA; note = Guide RNA targeting N-gene, DR rev, PFS = T
gaaacgtactacaccctttttgtaagggtctgaaaccgacattttgctctcaagctg

SEQ ID NO: 31 - RNA, 55 nt, synthetic construct
  source 1..55: mol_type = other RNA; note = Guide RNA targeting N-gene, DR dir, PFS = C
ggtttcagacccttacaaaaagggtgtagtacgtttccgcagtaaggatggctag

SEQ ID NO: 32 - RNA, 57 nt, synthetic construct
  source 1..57: mol_type = other RNA; note = Guide RNA targeting N-gene, DR rev, PFS = A
gaaacgtactacaccctttttgtaagggtctgaaacctaacgtacctgtctcttccg

SEQ ID NO: 33 - RNA, 57 nt, synthetic construct
  source 1..57: mol_type = other RNA; note = Guide RNA targeting N-gene, DR rev, PFS = T
gaaacgtactacaccctttttgtaagggtctgaaaccgtaaggatggctagtgtaac

SEQ ID NO: 34 - RNA, 58 nt, synthetic construct
  source 1..58: mol_type = other RNA; note = Guide RNA targeting N-gene, DR rev, PFS = G
gaaacgtactacaccctttttgtaagggtctgaaaccaatattgcagcagtacgcaca

SEQ ID NO: 35 - RNA, 59 nt, synthetic construct
  source 1..59: mol_type = other RNA; note = Guide RNA targeting N-gene, DR rev, PFS = C
gaaacgtactacaccctttttgtaagggtctgaaaccaagactcacgttaacaatattg

SEQ ID NO: 36 - RNA, 55 nt, synthetic construct
  source 1..55: mol_type = other RNA; note = Guide RNA targeting N-gene, DR rev, PFS = C
gaaacgtactacaccctttttgtaagggtctgaaacccgcagtaaggatggctag

SEQ ID NO: 37 - RNA, 20 nt, synthetic construct
  source 1..20: mol_type = other RNA; note = Guide domain of guide RNA targeting N-gene
ggtccaccaaacgtaatgcg

SEQ ID NO: 38 - RNA, 20 nt, synthetic construct
  source 1..20: mol_type = other RNA; note = Guide domain of guide RNA targeting N-gene
tctggttactgccagttgaa

SEQ ID NO: 39 - RNA, 20 nt, synthetic construct
  source 1..20: mol_type = other RNA; note = Guide domain of guide RNA targeting N-gene
tttgcggccaatgtttgtaa

SEQ ID NO: 40 - RNA, 20 nt, synthetic construct
  source 1..20: mol_type = other RNA; note = Guide domain of guide RNA targeting N-gene
ttggtgtattcaaggctccc

SEQ ID NO: 41 - RNA, 20 nt, synthetic construct
  source 1..20: mol_type = other RNA; note = Guide domain of guide RNA targeting N-gene
ggattgcgggtgccaatgtg

SEQ ID NO: 42 - RNA, 20 nt, synthetic construct
  source 1..20: mol_type = other RNA; note = Guide domain of guide RNA targeting N-gene
tgtagcacgattgcagcatt

SEQ ID NO: 43 - RNA, 20 nt, synthetic construct
  source 1..20: mol_type = other RNA; note = Guide domain of guide RNA targeting N-gene
tctagcaggagaagttcccc

SEQ ID NO: 44 - RNA, 20 nt, synthetic construct
  source 1..20: mol_type = other RNA; note = Guide domain of guide RNA targeting N-gene
tctgtcaagcagcagcaaag

SEQ ID NO: 45 - RNA, 20 nt, synthetic construct
  source 1..20: mol_type = other RNA; note = Guide domain of guide RNA targeting N-gene
gacattttgctctcaagctg

SEQ ID NO: 46 - RNA, 20 nt, synthetic construct
  source 1..20: mol_type = other RNA; note = Guide domain of guide RNA targeting N-gene
tggttactgccagttgaatc

SEQ ID NO: 47 - RNA, 21 nt, synthetic construct
  source 1..21: mol_type = other RNA; note = Guide domain of guide RNA targeting N-gene
aggattgcgggtgccaatgtg

SEQ ID NO: 48 - RNA, 21 nt, synthetic construct
  source 1..21: mol_type = other RNA; note = Guide domain of guide RNA targeting N-gene
ttgtagcacgattgcagcatt

SEQ ID NO: 49 - RNA, 23 nt, synthetic construct
  source 1..23: mol_type = other RNA; note = Guide domain of guide RNA targeting N-gene
caaattgtgcaatttgcggccaa

SEQ ID NO: 50 - RNA, 23 nt, synthetic construct
  source 1..23: mol_type = other RNA; note = Guide domain of guide RNA targeting N-gene
gccaatgtttgtaatcagttcct

SEQ ID NO: 51 - RNA, 23 nt, synthetic construct
  source 1..23: mol_type = other RNA; note = Guide domain of guide RNA targeting N-gene
ttgtctgattagttcctggtccc

SEQ ID NO: 52 - RNA, 18 nt, synthetic construct
  source 1..18: mol_type = other RNA; note = Guide domain of guide RNA targeting E-gene
cgcagtaaggatggctag

SEQ ID NO: 53 - RNA, 20 nt, synthetic construct
  source 1..20: mol_type = other RNA; note = Guide domain of guide RNA targeting E-gene
taacgtacctgtctcttccg

SEQ ID NO: 54 - RNA, 20 nt, synthetic construct
  source 1..20: mol_type = other RNA; note = Guide domain of guide RNA targeting E-gene
gtaaggatggctagtgtaac

SEQ ID NO: 55 - RNA, 21 nt, synthetic construct
  source 1..21: mol_type = other RNA; note = Guide domain of guide RNA targeting E-gene
aatattgcagcagtacgcaca

SEQ ID NO: 56 - RNA, 22 nt, synthetic construct
  source 1..22: mol_type = other RNA; note = Guide domain of guide RNA targeting E-gene
aagactcacgttaacaatattg

SEQ ID NO: 57 - RNA, 20 nt, synthetic construct
  source 1..20: mol_type = other RNA; note = N-gene Target sequence
cgcattacgtttggtggacc

SEQ ID NO: 58 - RNA, 20 nt, synthetic construct
  source 1..20: mol_type = other RNA; note = N-gene Target sequence
ttcaactggcagtaaccaga

SEQ ID NO: 59 - RNA, 20 nt, synthetic construct
  source 1..20: mol_type = other RNA; note = N-gene Target sequence
ttacaaacattggccgcaaa

SEQ ID NO: 60 - RNA, 20 nt, synthetic construct
  source 1..20: mol_type = other RNA; note = N-gene Target sequence
gggagccttgaatacaccaa

SEQ ID NO: 61 - RNA, 20 nt, synthetic construct
  source 1..20: mol_type = other RNA; note = N-gene Target sequence
cacattggcacccgcaatcc

SEQ ID NO: 62 - RNA, 20 nt, synthetic construct
  source 1..20: mol_type = other RNA; note = N-gene Target sequence
aatgctgcaatcgtgctaca

SEQ ID NO: 63 - RNA, 20 nt, synthetic construct
  source 1..20: mol_type = other RNA; note = N-gene Target sequence
ggggaacttctcctgctaga

SEQ ID NO: 64 - RNA, 20 nt, synthetic construct
  source 1..20: mol_type = other RNA; note = N-gene Target sequence
ctttgctgctgcttgacaga

SEQ ID NO: 65 - RNA, 20 nt, synthetic construct
  source 1..20: mol_type = other RNA; note = N-gene Target sequence
cagcttgagagcaaaatgtc

SEQ ID NO: 66 - RNA, 20 nt, synthetic construct
  source 1..20: mol_type = other RNA; note = N-gene Target sequence
gattcaactggcagtaacca

SEQ ID NO: 67 - RNA, 21 nt, synthetic construct
  source 1..21: mol_type = other RNA; note = N-gene Target sequence
cacattggcacccgcaatcct

SEQ ID NO: 68 - RNA, 21 nt, synthetic construct
  source 1..21: mol_type = other RNA; note = N-gene Target sequence
aatgctgcaatcgtgctacaa

SEQ ID NO: 69 - RNA, 23 nt, synthetic construct
  source 1..23: mol_type = other RNA; note = N-gene Target sequence
ttggccgcaaattgcacaatttg

SEQ ID NO: 70 - RNA, 23 nt, synthetic construct
  source 1..23: mol_type = other RNA; note = N-gene Target sequence
aggaactgattacaaacattggc

SEQ ID NO: 71 - RNA, 23 nt, synthetic construct
  source 1..23: mol_type = other RNA; note = N-gene Target sequence
gggaccaggaactaatcagacaa

SEQ ID NO: 72 - RNA, 18 nt, synthetic construct
  source 1..18: mol_type = other RNA; note = E-gene Target sequence
ctagccatccttactgcg

SEQ ID NO: 73 - RNA, 20 nt, synthetic construct
  source 1..20: mol_type = other RNA; note = E-gene Target sequence
cggaagagacaggtacgtta

SEQ ID NO: 74 - RNA, 20 nt, synthetic construct
  source 1..20: mol_type = other RNA; note = E-gene Target sequence
gttacactagccatccttac

SEQ ID NO: 75 - RNA, 21 nt, synthetic construct
  source 1..21: mol_type = other RNA; note = E-gene Target sequence
tgtgcgtactgctgcaatatt

SEQ ID NO: 76 - RNA, 22 nt, synthetic construct
  source 1..22: mol_type = other RNA; note = E-gene Target sequence
caatattgttaacgtgagtctt

SEQ ID NO: 77 - DNA, 60 bp, synthetic construct
  source 1..60: mol_type = other DNA; note = crRNA Forward primer
gaaattaatacgactcactataggaaacgtactacaccctttttgtaagggtctgaaacc

SEQ ID NO: 78 - DNA, 44 bp, synthetic construct
  source 1..44: mol_type = other DNA; note = crRNA Example 2.1 Reverse primer
gattcaactggcagtaaccaggtttcagacccttacaaaaaggg

SEQ ID NO: 79 - DNA, 45 bp, synthetic construct
  source 1..45: mol_type = other DNA; note = crRNA Example 2.2 Reverse primer
cacattggcacccgcaatcctggtttcagacccttacaaaaaggg

SEQ ID NO: 80 - DNA, 45 bp, synthetic construct
  source 1..45: mol_type = other DNA; note = crRNA Example 2.3 Reverse primer
aatgctgcaatcgtgctacaaggtttcagacccttacaaaaaggg

SEQ ID NO: 81 - DNA, 47 bp, synthetic construct
  source 1..47: mol_type = other DNA; note = crRNA Example 2.4 Reverse primer
ttggccgcaaattgcacaatttgggtttcagacccttacaaaaaggg

SEQ ID NO: 82 - DNA, 47 bp, synthetic construct
  source 1..47: mol_type = other DNA; note = crRNA Example 2.5 Reverse primer
aggaactgattacaaacattggcggtttcagacccttacaaaaaggg

SEQ ID NO: 83 - DNA, 47 bp, synthetic construct
  source 1..47: mol_type = other DNA; note = crRNA Example 2.6 Reverse primer
gggaccaggaactaatcagacaaggtttcagacccttacaaaaaggg

SEQ ID NO: 84 - DNA, 44 bp, synthetic construct
  source 1..44: mol_type = other DNA; note = crRNA Example 3.1 Reverse primer
cggaagagacaggtacgttaggtttcagacccttacaaaaaggg

SEQ ID NO: 85 - DNA, 44 bp, synthetic construct
  source 1..44: mol_type = other DNA; note = crRNA Example 3.2 Reverse primer
gttacactagccatccttacggtttcagacccttacaaaaaggg

SEQ ID NO: 86 - DNA, 45 bp, synthetic construct
  source 1..45: mol_type = other DNA; note = crRNA Example 3.3 Reverse primer
tgtgcgtactgctgcaatattggtttcagacccttacaaaaaggg

SEQ ID NO: 87 - DNA, 46 bp, synthetic construct
  source 1..46: mol_type = other DNA; note = crRNA Example 3.4 Reverse primer
caatattgttaacgtgagtcttggtttcagacccttacaaaaaggg